European Patent Application EP 4 446 419 A1, published October 16, 2024. Title: Recombinant adeno associated virus vector for treatment of neurodegeneration with brain iron accumulation. Applicant: Jichi-medical University. The sequence listing filed with the application follows.

SEQUENCE LISTING (9 sequences)

SEQ ID NO: 1 - protein, 360 aa, Homo sapiens
  REGION 1..360: note = MISC_FEATURE - WDR40 isoform 1 (w/o 1st Met)
TQQPLRGVTSLRFNQDQSCFCCAMETGVRIYNVEPLMEKGHLDHEQVGSMGLVEMLHRSNLLALVGGGSSPKFSEISAVLIWDDAREGKDSKEKLVLEFTFTKPVLSVRMRHDKIVIVLKNRIYVYSFPDNPRKLFEFDTRDNPKGLCDLCPSLEKQLLVFPGHKCGSLQLVDLASTKPGTSSAPFTINAHQSDIACVSLNQPGTVVASASQKGTLIRLFDTQSKEKLVELRRGTDPATLYCINFSHDSSFLCASSDKGTVHIFALKDTRLNRRSALARVGKVGPMIGQYVDSQWSLASFTVPAESACICAFGRNTSKNVNSVIAICVDGTFHKYVFTPDGNCNREAFDVYLDICDDDDF

SEQ ID NO: 2 - protein, 359 aa, Homo sapiens
  REGION 1..359: note = MISC_FEATURE - WDR40 isoform 2 (w/o 1st Met)
TQQPLRGVTSLRFNQDQSCFCCAMETGVRIYNVEPLMEKGHLDHEQVGSMGLVEMLHRSNLLALVGGGSSPKFSEISVLIWDDAREGKDSKEKLVLEFTFTKPVLSVRMRHDKIVIVLKNRIYVYSFPDNPRKLFEFDTRDNPKGLCDLCPSLEKQLLVFPGHKCGSLQLVDLASTKPGTSSAPFTINAHQSDIACVSLNQPGTVVASASQKGTLIRLFDTQSKEKLVELRRGTDPATLYCINFSHDSSFLCASSDKGTVHIFALKDTRLNRRSALARVGKVGPMIGQYVDSQWSLASFTVPAESACICAFGRNTSKNVNSVIAICVDGTFHKYVFTPDGNCNREAFDVYLDICDDDDF

SEQ ID NO: 3 - protein, 650 aa, Homo sapiens
  REGION 1..650: note = MISC_FEATURE - human NCOA4 isoform 1
MGAQLTTFALAGAVRRMNTFQDQSGSSSNREPLLRCSDARRDLELAIGGVLRAEQQIKDNLREVKAQIHSCISRHLECLRSREVWLYEQVDLIYQLKEETLQQQAQQLYSLLGQFNCLTHQLECTQNKDLANQVSVCLERLGSLTLKPEDSTVLLFEADTITLRQTITTFGSLKTIQIPEHLMAHASSANIGPFLEKRGCISMPEQKSASGIVAVPFSEWLLGSKPASGYQAPYIPSTDPQDWLTQKQTLENSQTSSRACNFFNNVGGNLKGLENWLLKSEKSSYQKCNSHSTTSSFSIEMEKVGDQELPDQDEMDLSDWLVTPQESHKLRKPENGSRETSEKFKLLFQSYNVNDWLVKTDSCTNCQGNQPKGVEIENLGNLKCLNDHLEAKKPLSTPSMVTEDWLVQNHQDPCKVEEVCRANEPCTSFAECVCDENCEKEALYKWLLKKEGKDKNGMPVEPKPEPEKHKDSLNMWLCPRKEVIEQTKAPKAMTPSRIADSFQVIKNSPLSEWLIRPPYKEGSPKEVPGTEDRAGKQKFKSPMNTSWCSFNTADWVLPGKKMGNLSQLSSGEDKWLLRKKAQEVLLNSPLQEEHNFPPDHYGLPAVCDLFACMQLKVDKEKWLYRTPLQAYFKMNFQDVTVGNFQIPCGF

SEQ ID NO: 4 - protein, 630 aa, Homo sapiens
  REGION 1..630: note = MISC_FEATURE - human NCOA4 isoform 2
MGAQLTTFALAGAVRRMNTFQDQSGSSSNREPLLRCSDARRDLELAIGGVLRAEQQIKDNLREVKAQIHSCISRHLECLRSREVWLYEQVDLIYQLKEETLQQQAQQLYSLLGQFNCLTHQLECTQNKDLANQVSVCLERLGSLTLKPEDSTVLLFEADTITLRQTITTFGSLKTIQIPEHLMAHASSANIGPFLEKRGCISMPEQKSASGIVAVPFSEWLLGSKPASGYQAPYIPSTDPQDWLTQKQTLENSQTSSRACNFFNNVGGNLKGLENWLLKSEKSSYQKCNSHSTTSSFSIEMEKVGDQELPDQDEMDLSDWLVTPQESHKLRKPENGSRETSEKFKLLFQSYNVNDWLVKTDSCTNCQGNQPKGVEIENLGNLKCLNDHLEAKKPLSTPSMVTEDWLVQNHQDPCKVEEVCRANEPCTSFAECVCDENCEKEALYKWLLKKEGKDKNGMPVEPKPEPEKHKDSLNMWLCPRKEVIEQTKAPKAMTPSRIADSFQVIKNSPLSEWLIRPPYKEGSPKEVPGTEDRAGKQKFKSPMNTSWCSFNTADWVLPGKKMGNLSQLSSGEDKWLLRKKAQEVLLNSPLQEEHNFPPDHYGLPAVCDLFACMQLKVDKEKWLYRTPLQM

SEQ ID NO: 5 - protein, 614 aa, Homo sapiens
  REGION 1..614: note = MISC_FEATURE - human NCOA4 isoform 3
MNTFQDQSGSSSNREPLLRCSDARRDLELAIGGVLRAEQQIKDNLREVKAQIHSCISRHLECLRSREVWLYEQVDLIYQLKEETLQQQAQQLYSLLGQFNCLTHQLECTQNKDLANQVSVCLERLGSLTLKPEDSTVLLFEADTITLRQTITTFGSLKTIQIPEHLMAHASSANIGPFLEKRGCISMPEQKSASGIVAVPFSEWLLGSKPASGYQAPYIPSTDPQDWLTQKQTLENSQTSSRACNFFNNVGGNLKGLENWLLKSEKSSYQKCNSHSTTSSFSIEMEKVGDQELPDQDEMDLSDWLVTPQESHKLRKPENGSRETSEKFKLLFQSYNVNDWLVKTDSCTNCQGNQPKGVEIENLGNLKCLNDHLEAKKPLSTPSMVTEDWLVQNHQDPCKVEEVCRANEPCTSFAECVCDENCEKEALYKWLLKKEGKDKNGMPVEPKPEPEKHKDSLNMWLCPRKEVIEQTKAPKAMTPSRIADSFQVIKNSPLSEWLIRPPYKEGSPKEVPGTEDRAGKQKFKSPMNTSWCSFNTADWVLPGKKMGNLSQLSSGEDKWLLRKKAQEVLLNSPLQEEHNFPPDHYGLPAVCDLFACMQLKVDKEKWLYRTPLQM

SEQ ID NO: 6 - protein, 575 aa, Homo sapiens
  REGION 1..575: note = MISC_FEATURE - human NCOA4 (575aa version)
MNTFQDQSGSSSNREPLLRCSDARRDLELAIGGVLRAEQQIKDNLREVKAQIHSCISRHLECLRSREVWLYEQVDLIYQLKEETLQQQAQQLYSLLGQFNCLTHQLECTQNKDLANQVSVCLERLGSLTLKPEDSTVLLFEADTITLRQTITTFGSLKTIQIPEHLMAHASSANIGPFLEKRGCISMPEQKSASGIVAVPFSEWLLGSKPASGYQAPYIPSTDPQDWLTQKQTLENSQTSSRACNFFNNVGGNLKGLENWLLKSEKSSYQKCNSHSTTSSFSIEMEKVGDQELPDQDEMDLSDWLVTPQESHKLRKPENGSRETSEKFKLLFQSYNVNDWLVKTDSCTNCQGNQPKGVEIENLGNLKCLNDHLEAKKPLSTPSMVTEDWLVQNHQDPCKVEEVCRANEPCTSFAECVCDENCEKEALYKWLLKKEGKDKNGMPVEPKPEPEKHKDSLNMWLCPRKEVIEQTKAPKAMTPSRIADSFQVIKNSPLSEWLIRPPYKEGSPKEVPGTEDRAGKQKYYLIHLYRRNITSPQTIMASLQFVISLPVCSLKLIKRSGYIELLYRCEGMDKS

SEQ ID NO: 7 - protein, 735 aa, synthetic construct
  REGION 1..735: note = AAV1 VP1(Y445F)(w/o 1st Met)
AADGYLPDWLEDNLSEGIREWWDLKPGAPKPKANQQKQDDGRGLVLPGYKYLGPFNGLDKGEPVNAADAAALEHDKAYDQQLKAGDNPYLRYNHADAEFQERLQEDTSFGGNLGRAVFQAKKRVLEPLGLVEEGAKTAPGKKRPVEQSPQEPDSSSGIGKTGQQPAKKRLNFGQTGDSESVPDPQPLGEPPATPAAVGPTTMASGGGAPMADNNEGADGVGNASGNWHCDSTWLGDRVITTSTRTWALPTYNNHLYKQISSASTGASNDNHYFGYSTPWGYFDFNRFHCHFSPRDWQRLINNNWGFRPKRLNFKLFNIQVKEVTTNDGVTTIANNLTSTVQVFSDSEYQLPYVLGSAHQGCLPPFPADVFMIPQYGYLTLNNGSQAVGRSSFYCLEYFPSQMLRTGNNFTFSYTFEEVPFHSSYAHSQSLDRLMNPLIDQYLYFLNRTQNQSGSAQNKDLLFSRGSPAGMSVQPKNWLPGPCYRQQRVSKTKTDNNNSNFTWTGASKYNLNGRESIINPGTAMASHKDDEDKFFPMSGVMIFGKESAGASNTALDNVMITDEEEIKATNPVATERFGTVAVNFQSSSTDPATGDVHAMGALPGMVWQDRDVYLQGPIWAKIPHTDGHFHPSPLMGGFGLKNPPPQILIKNTPVPANPPAEFSATKFASFITQYSTGQVSVEIEWELQKENSKRWNPEVQYTSNYAKSANVDFTVDNNGLYTEPRPIGTRYLTRPL

SEQ ID NO: 8 - protein, 734 aa, synthetic construct
  REGION 1..734: note = AAV2 VP1(Y444F)(w/o 1st Met)
AADGYLPDWLEDTLSEGIRQWWKLKPGPPPPKPAERHKDDSRGLVLPGYKYLGPFNGLDKGEPVNEADAAALEHDKAYDRQLDSGDNPYLKYNHADAEFQERLKEDTSFGGNLGRAVFQAKKRVLEPLGLVEEPVKTAPGKKRPVEHSPVEPDSSSGTGKAGQQPARKRLNFGQTGDADSVPDPQPLGQPPAAPSGLGTNTMATGSGAPMADNNEGADGVGNSSGNWHCDSTWMGDRVITTSTRTWALPTYNNHLYKQISSQSGASNDNHYFGYSTPWGYFDFNRFHCHFSPRDWQRLINNNWGFRPKRLNFKLFNIQVKEVTQNDGTTTIANNLTSTVQVFTDSEYQLPYVLGSAHQGCLPPFPADVFMVPQYGYLTLNNGSQAVGRSSFYCLEYFPSQMLRTGNNFTFSYTFEDVPFHSSYAHSQSLDRLMNPLIDQYLYFLSRTNTPSGTTTQSRLQFSQAGASDIRDQSRNWLPGPCYRQQRVSKTSADNNNSEYSWTGATKYHLNGRDSLVNPGPAMASHKDDEEKFFPQSGVLIFGKQGSEKTNVDIEKVMITDEEEIRTTNPVATEQYGSVSTNLQRGNRQAATADVNTQGVLPGMVWQDRDVYLQGPIWAKIPHTDGHFHPSPLMGGFGLKHPPPQILIKNTPVPANPSTTFSAAKFASFITQYSTGQVSVEIEWELQKENSKRWNPEIQYTSNYNKSVNVDFTVDTNGVYSEPRPIGTRYLTRNL

SEQ ID NO: 9 - protein, 735 aa, synthetic construct
  REGION 1..735: note = AAV9 VP1(Y446F)(w/o 1st Met)
AADGYLPDWLEDNLSEGIREWWALKPGAPQPKANQQHQDNARGLVLPGYKYLGPGNGLDKGEPVNAADAAALEHDKAYDQQLKAGDNPYLKYNHADAEFQERLKEDTSFGGNLGRAVFQAKKRLLEPLGLVEEAAKTAPGKKRPVEQSPQEPDSSAGIGKSGAQPAKKRLNFGQTGDTESVPDPQPIGEPPAAPSGVGSLTMASGGGAPVADNNEGADGVGSSSGNWHCDSQWLGDRVITTSTRTWALPTYNNHLYKQISNSTSGGSSNDNAYFGYSTPWGYFDFNRFHCHFSPRDWQRLINNNWGFRPKRLNFKLFNIQVKEVTDNNGVKTIANNLTSTVQVFTDSDYQLPYVLGSAHEGCLPPFPADVFMIPQYGYLTLNDGSQAVGRSSFYCLEYFPSQMLRTGNNFQFSYEFENVPFHSSYAHSQSLDRLMNPLIDQYLYFLSKTINGSGQNQQTLKFSVAGPSNMAVQGRNYIPGPSYRQQRVSTTVTQNNNSEFAWPGASSWALNGRNSLMNPGPAMASHKEGEDRFFPLSGSLIFGKQGTGRDNVDADKVMITNEEEIKTTNPVATESYGQVATNHQSAQAQAQTGWVQNQGILPGMVWQDRDVYLQGPIWAKIPHTDGNFHPSPLMGGFGMKHPPPQILIKNTPVPADPPTAFNKDKLNSFITQYSTGQVSVEIEWELQKENSKRWNPEIQYTSNYYKSNNVEFAVNTEGVYSEPRPIGTRYLTRNL